European Patent Specification EP 3 699 298 B1, published April 24, 2024. Title: COMPOSITIONS AND METHODS FOR DETECTING A BIOLOGICAL CONTAMINANT. Applicant: Regeneron Pharmaceuticals, Inc. Application PCT/US16/24216. The sequence listing filed with the application follows.

SEQUENCE LISTING (37 sequences)

SEQ ID NO: 1 - DNA, 24 bp, Parvovirus
tgcataaaagagtaacctcaccag

SEQ ID NO: 2 - DNA, 18 bp, Parvovirus
actggatgatgatgcagc

SEQ ID NO: 3 - DNA, 19 bp, Parvovirus
tgtcgatggcgaatggcta

SEQ ID NO: 4 - DNA, 18 bp, Parvovirus
ccacctggttgagccatc

SEQ ID NO: 5 - DNA, 20 bp, Bacteriophage M13
aagcctcagcgaccgaatat

SEQ ID NO: 6 - DNA, 24 bp, Bacteriophage M13
tatgcgtgggcgatggttgttgtc

SEQ ID NO: 7 - DNA, 22 bp, Bacteriophage M13
tcagcttgctttcgaggtgaat

SEQ ID NO: 8 - DNA, 6407 bp, Bacteriophage M13
aacgctactactattagtagaattgatgccaccttttcagctcgcgccccaaatgaaaatatagctaaacaggttattgaccatttgcgaaatgtatctaatggtcaaactaaatctactcgttcgcagaattgggaatcaactgttacatggaatgaaacttccagacaccgtactttagttgcatatttaaaacatgttgagctacagcaccagattcagcaattaagctctaagccatccgcaaaaatgacctcttatcaaaaggagcaattaaaggtactctctaatcctgacctgttggagtttgcttccggtctggttcgctttgaagctcgaattaaaacgcgatatttgaagtctttcgggcttcctcttaatctttttgatgcaatccgctttgcttctgactataatagtcagggtaaagacctgatttttgatttatggtcattctcgttttctgaactgtttaaagcatttgagggggattcaatgaatatttatgacgattccgcagtattggacgctatccagtctaaacattttactattaccccctctggcaaaacttcttttgcaaaagcctctcgctattttggtttttatcgtcgtctggtaaacgagggttatgatagtgttgctcttactatgcctcgtaattccttttggcgttatgtatctgcattagttgaatgtggtattcctaaatctcaactgatgaatctttctacctgtaataatgttgttccgttagttcgttttattaacgtagatttttcttcccaacgtcctgactggtataatgagccagttcttaaaatcgcataaggtaattcacaatgattaaagttgaaattaaaccatctcaagcccaatttactactcgttctggtgtttctcgtcagggcaagccttattcactgaatgagcagctttgttacgttgatttgggtaatgaatatccggttcttgtcaagattactcttgatgaaggtcagccagcctatgcgcctggtctgtacaccgttcatctgtcctctttcaaagttggtcagttcggttcccttatgattgaccgtctgcgcctcgttccggctaagtaacatggagcaggtcgcggatttcgacacaatttatcaggcgatgatacaaatctccgttgtactttgtttcgcgcttggtataatcgctgggggtcaaagatgagtgttttagtgtattctttcgcctctttcgttttaggttggtgccttcgtagtggcattacgtattttacccgtttaatggaaacttcctcatgaaaaagtctttagtcctcaaagcctctgtagccgttgctaccctcgttccgatgctgtctttcgctgctgagggtgacgatcccgcaaaagcggcctttaactccctgcaagcctcagcgaccgaatatatcggttatgcgtgggcgatggttgttgtcattgtcggcgcaactatcggtatcaagctgtttaagaaattcacctcgaaagcaagctgataaaccgatacaattaaaggctccttttggagcctttttttttggagattttcaacatgaaaaaattattattcgcaattcctttagttgttcctttctattctcactccgctgaaactgttgaaagttgtttagcaaaaccccatacagaaaattcatttactaacgtctggaaagacgacaaaactttagatcgttacgctaactatgagggttgtctgtggaatgctacaggcgttgtagtttgtactggtgacgaaactcagtgttacggtacatgggttcctattgggcttgctatccctgaaaatgagggtggtggctctgagggtggcggttctgagggtggcggttctgagggtggcggtactaaacctcctgagtacggtgatacacctattccgggctatacttatatcaaccctctcgacggcacttatccgcctggtactgagcaaaaccccgctaatcctaatccttctcttgaggagtctcagcctcttaatactttcatgtttcagaataataggttccgaaataggcagggggcattaactgtttatacgggcactgttactcaaggcactgaccccgttaaaacttattaccagtacactcctgtatcatcaaaagccatgtatgacgcttactggaacggtaaattcagagactgcgctttccattctggctttaatgaggatccattcgtttgtgaatatcaaggccaatcgtctgacctgcctcaacctcctgtcaatgctggcggcggctctggtggtggttctggtggcggctctgagggtggtggctctgagggtggcggttctgagggtggcggctctgagggaggcggttccggtggtggctctggttccggtgattttgattatgaaaagatggcaaacgctaataagggggctatgaccgaaaatgccgatgaaaacgcgctacagtctgacgctaaaggcaaacttgattctgtcgctactgattacggtgctgctatcgatggtttcattggtgacgtttccggccttgctaatggtaatggtgctactggtgattttgctggctctaattcccaaatggctcaagtcggtgacggtgataattcacctttaatgaataatttccgtcaatatttaccttccctccctcaatcggttgaatgtcgcccttttgtctttagcgctggtaaaccatatgaattttctattgattgtgacaaaataaacttattccgtggtgtctttgcgtttcttttatatgttgccacctttatgtatgtattttctacgtttgctaacatactgcgtaataaggagtcttaatcatgccagttcttttgggtattccgttattattgcgtttcctcggtttccttctggtaactttgttcggctatctgcttacttttcttaaaaagggcttcggtaagatagctattgctatttcattgtttcttgctcttattattgggcttaactcaattcttgtgggttatctctctgatattagcgctcaattaccctctgactttgttcagggtgttcagttaattctcccgtctaatgcgcttccctgtttttatgttattctctctgtaaaggctgctattttcatttttgacgttaaacaaaaaatcgtttcttatttggattgggataaataatatggctgtttattttgtaactggcaaattaggctctggaaagacgctcgttagcgttggtaagattcaggataaaattgtagctgggtgcaaaatagcaactaatcttgatttaaggcttcaaaacctcccgcaagtcgggaggttcgctaaaacgcctcgcgttcttagaataccggataagccttctatatctgatttgcttgctattgggcgcggtaatgattcctacgatgaaaataaaaacggcttgcttgttctcgatgagtgcggtacttggtttaatacccgttcttggaatgataaggaaagacagccgattattgattggtttctacatgctcgtaaattaggatgggatattatttttcttgttcaggacttatctattgttgataaacaggcgcgttctgcattagctgaacatgttgtttattgtcgtcgtctggacagaattactttaccttttgtcggtactttatattctcttattactggctcgaaaatgcctctgcctaaattacatgttggcgttgttaaatatggcgattctcaattaagccctactgttgagcgttggctttatactggtaagaatttgtataacgcatatgatactaaacaggctttttctagtaattatgattccggtgtttattcttatttaacgccttatttatcacacggtcggtatttcaaaccattaaatttaggtcagaagatgaaattaactaaaatatatttgaaaaagttttctcgcgttctttgtcttgcgattggatttgcatcagcatttacatatagttatataacccaacctaagccggaggttaaaaaggtagtctctcagacctatgattttgataaattcactattgactcttctcagcgtcttaatctaagctatcgctatgttttcaaggattctaagggaaaattaattaatagcgacgatttacagaagcaaggttattcactcacatatattgatttatgtactgtttccattaaaaaaggtaattcaaatgaaattgttaaatgtaattaattttgttttcttgatgtttgtttcatcatcttcttttgctcaggtaattgaaatgaataattcgcctctgcgcgattttgtaacttggtattcaaagcaatcaggcgaatccgttattgtttctcccgatgtaaaaggtactgttactgtatattcatctgacgttaaacctgaaaatctacgcaatttctttatttctgttttacgtgctaataattttgatatggttggttcaattccttccataattcagaagtataatccaaacaatcaggattatattgatgaattgccatcatctgataatcaggaatatgatgataattccgctccttctggtggtttctttgttccgcaaaatgataatgttactcaaacttttaaaattaataacgttcgggcaaaggatttaatacgagttgtcgaattgtttgtaaagtctaatacttctaaatcctcaaatgtattatctattgacggctctaatctattagttgttagtgcacctaaagatattttagataaccttcctcaattcctttctactgttgatttgccaactgaccagatattgattgagggtttgatatttgaggttcagcaaggtgatgctttagatttttcatttgctgctggctctcagcgtggcactgttgcaggcggtgttaatactgaccgcctcacctctgttttatcttctgctggtggttcgttcggtatttttaatggcgatgttttagggctatcagttcgcgcattaaagactaatagccattcaaaaatattgtctgtgccacgtattcttacgctttcaggtcagaagggttctatctctgttggccagaatgtcccttttattactggtcgtgtgactggtgaatctgccaatgtaaataatccatttcagacgattgagcgtcaaaatgtaggtatttccatgagcgtttttcctgttgcaatggctggcggtaatattgttctggatattaccagcaaggccgatagtttgagttcttctactcaggcaagtgatgttattactaatcaaagaagtattgctacaacggttaatttgcgtgatggacagactcttttactcggtggcctcactgattataaaaacacttctcaagattctggcgtaccgttcctgtctaaaatccctttaatcggcctcctgtttagctcccgctctgattccaacgaggaaagcacgttatacgtgctcgtcaaagcaaccatagtacgcgccctgtagcggcgcattaagcgcggcgggtgtggtggttacgcgcagcgtgaccgctacacttgccagcgccctagcgcccgctcctttcgctttcttcccttcctttctcgccacgttcgccggctttccccgtcaagctctaaatcgggggctccctttagggttccgatttagtgctttacggcacctcgaccccaaaaaacttgatttgggtgatggttcacgtagtgggccatcgccctgatagacggtttttcgccctttgacgttggagtccacgttctttaatagtggactcttgttccaaactggaacaacactcaaccctatctcgggctattcttttgatttataagggattttgccgatttcggcctattggttaaaaaatgagctgatttaacaaaaatttaacgcgaattttaacaaaatattaacgtttacaatttaaatatttgcttatacaatcttcctgtttttggggcttttctgattatcaaccggggtacatatgattgacatgctagttttacgattaccgttcatcgattctcttgtttgctccagactctcaggcaatgacctgatagcctttgtagacctctcaaaaatagctaccctctccggcatgaatttatcagctagaacggttgaatatcatattgatggtgatttgactgtctccggcctttctcacccttttgaatctttacctacacattactcaggcattgcatttaaaatatatgagggttctaaaaatttttatccttgcgttgaaataaaggcttctcccgcaaaagtattacagggtcataatgtttttggtacaaccgatttagctttatgctctgaggctttattgcttaattttgctaattctttgccttgcctgtatgatttattggatgtt

SEQ ID NO: 9 - DNA, 2019 bp, Minute virus of mouse
atggctggaaatgcttactctgatgaagttttgggagcaaccaactggttaaaggaaaaaagtaaccaggaagtgttctcatttgtttttaaaaatgaaaatgttcaactgaatggaaaagatatcggatggaatagttacaaaaaagagctgcaggaggacgagctgaaatctttacaacgaggagcggaaactacttgggaccaaagcgaggacatggaatgggaaaccacagtggatgaaatgaccaaaaagcaagtattcatttttgattctttggttaaaaaatgtttatttgaagtgcttaacacaaagaatatatttcctggtgatgttaattggtttgtgcaacatgaatggggaaaagaccaaggctggcactgccatgtactaattggaggaaaggactttagtcaagctcaagggaaatggtggagaaggcaactaaatgtttactggagcagatggttggtaacagcctgtaatgtgcaactaacaccagctgaaagaattaaactaagagaaatagcagaagacaatgagtgggttactctacttacttataagcataagcaaaccaaaaaagactataccaagtgtgttctttttggaaacatgattgcttactattttttaactaaaaagaaaataagcactagtccaccaagagacggaggctattttcttagcagtgactctggctggaaaactaactttttaaaagaaggcgagcgccatctagtgagcaaactatacactgatgacatgcggccagaaacggttgaaaccacagtaaccactgcgcaggaaactaagcgcggcagaattcaaactaaaaaagaagtttctattaaaactacacttaaagagctggtgcataaaagagtaacctcaccagaggactggatgatgatgcagccagacagttacattgaaatgatggctcaaccaggtggagaaaacctgctgaaaaatacgctagagatttgtacactaactctagccagaaccaaaacagcatttgacttaattttagaaaaagctgaaaccagcaaactaaccaacttttcactgcctgacacaagaacctgcagaatttttgcttttcatggctggaactatgttaaagtttgccatgctatttgctgtgttttaaacagacaaggaggcaaaagaaatactgttttatttcatggaccagccagcacaggcaaatctattattgcacaagccatagcacaagcagttggcaatgttggttgctataatgcagccaatgtaaactttccatttaatgactgtaccaacaagaacttgatttgggtagaagaagctggtaactttggacagcaagtaaaccagtttaaagccatttgctctggtcaaactattcgcattgatcaaaaaggaaaaggcagcaaacagattgaaccaacaccagtcatcatgaccacaaatgagaacattacagtggtcagaataggctgcgaagaaagaccagaacacactcaaccaatcagagacagaatgcttaacattcatctaacacataccttgcctggtgactttggtttggttgacaaaaatgaatggcccatgatttgtgcttggttggtaaagaatggttaccaatctaccatggcaagctactgtgctaaatggggcaaagttcctgattggtcagaaaactgggcggagccaaaggtgccaactcctataaatttactaggttcggcacgctcaccattcacgacaccgaaaagtacgcctctcagccagaactatgcactaactccacttgcatcggatctcgaggacctggctttagagccttggagcacaccaaatactcctgttgcgggcactgcagaaacccagaacactggggaagctggttccaaagcctgccaagatggtcaactgagcccaacttggtcagagatcgaggaggatttgagagcgtgcttcggtgcggaaccgttgaagaaagacttcagcgagccgctgaacttggactaa

SEQ ID NO: 10 - DNA, 19 bp, Artificial
  synthetic
tagccattcgccatcgaca

SEQ ID NO: 11 - DNA, 1707 bp, Artificial
  synthetic
aagcctcagcgaccgaatatatcggttatgcgtgggcgatggttgttgtcattgtcggcgcaactatcggtatcaagctgtttaagaaattcacctcgaaagcaagctgacacgcctaccgcgatgctgaatgacccggactagagtggcgaaatttatggcgtgtgacccgttatgctccatttcggtcagtgggtcattgctagtagtcgattgcattgccattctccgagtgatttagcgtgacagccgcagggaacccataaaatgcaatcgtagtccacctgatcgtacttagaaatgagggtccccttttgcccacgcacctgttcgctcgtcgtttgcttttaagaaccgcacgaaccacagagcataaagagaacctctagctcctttacaaggtactggttccctttccagcgggatgccttatctaaacgcaatgacagacgtattcctcaggccacatcgcttcctacttccgctgggatccatcattggcggccgaagccgccattccatagtgagtccttcgtctgtgtctttctgtgccagatcgtctagcaaattgccgatccagtttatctcacgaaactatagtcgtacagaccgaaatcttaagtcaaatcacgcgactaggctcagctctattttagtggtcatgggttttggtccgcccgagcggtgcaaccgattaggaccatgtaaaacatttgttacaagtcttcttttaaacacaatcttcctgctcagtggcgcatgattatcgttgttgctagccagcgtggtaagtaacagcaccactgcgagcctaatgtgccctttccacgaacacagggctgtccgatcctatattaggactccgcaatggggttagcaagtcgcaccctaaacgatgttgaagactcgcgatgtacatgctctggtacaatacatacgtgttccggctgttatcctgcatcggaacctcaatcatgcatcgcaccagcgtattcgtgtcatctaggaggggcgcgtaggataaataattcaattaagatgtcgttatgctagtatacgcctacccgtcaccggccatctgtgtgcagatggggcgacgagttactggccctgatttctccgcttctaataccacacactgggcaatacgagctcaagccagtctcgcagtaacgctcatcagctaacgaaagagttagaggctcgctaacggagacgagttaaagacacgagttcccaaaaccaggcgggctcgccacgacggctaatcctggtagtttacgtgaacaatgttctgaagaaaatttgtgaaagaaggacccgtcaccgcctacaattacctacaacggtcggccgcaccttcgattgtcgtggccaccctcggattacacggcagaggtggttgtgtcccgacaggccagcatattatcctgaggcgttaccccaatcgttctccgtcggatttgctacagcccctgagcgctacatgcacgaaaccaagttatgtatgcactgggccgtcaataggacgtagccttgtagttagcacgtagcccggccgcattagtacagtagagcctccgccggcatcctgtttattaagttatttctgcataaaagagtaacctcaccagaggactggatgatgatgcagccagacagttagccattcgccatcgacattgaaatgatggctcaaccaggtgg

SEQ ID NO: 12 - DNA, 2019 bp, Mvm lymphotropic variant
atggctggaaatgcttactctgatgaagttttgggaacaaccaactggttaaaggaaaaaagtaaccaggaagtgttctcatttgtttttaaaactgaggatgttcaactaaatggaaaagatatcggatggaataattacaaaaaggagctgcaggaggacgagctgaaatctttacaacgaggagcggaaactacctgggaccaaagcgaggacatggaatgggaatctacagtggatgaaatgaccaaaaagcaagtattcatttatgactctttagttaaaaaatgtttgtttgaagtgcttagcacaaaaaatatagctcctgctgatgttacttggtttgtgcagcatgaatgggggaaagaccaaggctggcactgccatgtactaattggaggcaaggactttagtcaagctcaaggaaaatggtggagaaggcagctaaatgtttactggagcagatggttggtaacagcctgtaatgtgcagctaacaccagctgaaagaattaaactaagagaaatagcagaagacagtgagtgggttactttactcacttataaacataagcaaaccaaaaaggactatactaaatgtgttctttttggaaatatgattgcttactactttttaaccaaaaagaaaataagcaccagtccgccaagggacggaggctattttctaagcagtgactctggctggaaaactaactttttaaaagagggcgaacgccatctagtgagcaaattatacactgatgacatgcggccagaaacggttgaaaccacagtaaccactgcgcaggaaactaagcgcggcagaattcaaactaaaaaagaggtttctattaaaaccacacttaaagagctagtgcataaaagagtaacctcaccagaagactggatgatgatgcagccagacagttacattgaaatgatggctcaaccaggtggagaaaacctgctgaaaaatacgctagagatttgtacgctaactctagccagaacaaaaacagcatttgacttgattttagaaaaagctgaaaccagcaaactaaccaacttttcactgcctgacacaagaacctgcaagatttttgcttttcatggctggaactatgttaaagtttgccatgctatttgctgtgttctaaacagacaaggaggcaaaagaaatactgttttatttcacggaccagccagtacaggcaaatctattattgcacaagccatagcacaggcagttggtaatgttggttgctataatgcagctaatgtgaactttccatttaatgactgtaccaacaagaacttgatttgggtagaagaagctggtaactttggacagcaagtaaaccagtttaaagccatttgctctggtcaaactattcgcattgatcaaaaaggaaaaggcagcaaacaaattgaaccaacaccagtcatcatgaccacaaatgagaacattacagtggtcagaataggctgcgaagagagaccagaacacactcaaccaattagagacagaatgctcaacattcatctaacacatacattgcctggtgactttggtttggttgacaagaatgaatggcccatgatttgtgcttggttggtaaagaatggttaccaatctaccatggcaagctactgcgctaaatggggcaaagttcctgattggtcagaaaactgggcggagccaaaggtgccgactcctataaattcactaggttcggcacgctcaccattcacgacaccgaaaagtacgcctctcagccagaactatgcaataactccacttgcatcggatctcgaggacctggctttagagccttggagcacaccaaatactcctgttgcgggcactgcagaaacccagaacactggggaagctggttccaaagcctgccaagatggtcaactgagcccaacttggtcagagatcgaggaggatttgagagcgtgcttcggtgcggaaccgttgaagagagacttcagcgagccgctgaacttggactaa

SEQ ID NO: 13 - DNA, 2019 bp, Mouse parvovirus 4b
atggctggaaatgcttactctgatgaagttttgggagcaaccaactggttaaaggaaaaaagtaaccaggaagtattctcatttgtttttaaaaatgaggatgttcaactgaatggaaaagatattggatggaatagctacaaaaaagagctacaggaggacgagctgaaatctttacaacgaggagcggaaactacctgggaccaaagcgaggacatggaatgggaatctacagtggatgaagtaaccaaaaagcaagtattcatttttgactctttagttaaaaaatgtttgtttgaagtgcttaacacaaagaacatagctcctagtgatgttaattggtttgtacagcatgaatggggaaaagaccaaggctggcattgccatgtactaattggaggcaaagactttagtcaagctcaaggaaagtggtggagaaggcagctaaatgtttactggagcagatggttggtaacagcctgtaatgtgcagctatcaccagctgaaagaattaaactaagagaaatagcagaagacaatgagtgggttagcttgctcacttataagcataagcaaaccaaaaaggactatactaagtgtgttctttttggcaacatgattgcttactactttttaaccaaaaagaaaataagcactagtccaccaagggacggaggctattttctaagcagtgactctggctggaaaactaactttttaaaagaaggcgaacgccatctagtgagcaaactatacactgatgacatgcggccagaaacggttgaaaccacagtaaccactgcacaggaaactaagcgcggcagaattcaaactaaaaaagaggtttctattaaaaccacacttaaagagctggtgcataaaagagtaacctcaccagaagactggatgatgatgcagccagacagttatattgaaatgatggctcaaccaggtggagaaaacctgctgaaaaatacgctagagatttgtacactaactctagctagaaccaaaacagcatttgacttgattttagaaaaagctgaaaccagcaaactaactaacttttcactgccggacacaagaacctgcaagatttttgcttttcatggctggaactacattaaagtttgccatgctatttgctgtgttttaaacagacaaggaggcaaaagaaatactgttttatttcatggaccagccagtacaggcaaatccattattgcacaagccatagcacaggcagttggtaatgttggttgctataatgcagcaaatgtaaactttccattcaatgactgtaccaacaagaacttgatttgggtggaagaagctggtaactttggacagcaagtaaaccagttcaaagccatttgctctggtcaaactattcgcattgatcaaaaaggaaaaggcagcaaacagattgaaccaacaccagtcatcatgaccacaaatgaaaacattacagtggtcagaataggctgtgaagaaagaccagagcacactcaaccaatcagagacagaatgcttaacattcatctaacacatacattgcctggtgactttggtttggttgacaaaaatgagtggcccatgatttgtgcttggttggtaaagaatggttaccaatctaccatggcaagctactgtgctaaatggggcaaagttcctgattggacggaaaactgggcggagccgaaggtgccgactcctataaattcactaggttcggcacgctcaccattcacgacaccgaaaagtacgcctctcagccagaactatgcactaactccacttgcatcggatctcgaggacctggctttagagccttggagcacaccaaatactcctgttgtgggcactgcagaaacccagaacactggggaagctggttccaaagcctgccaagatggtcaactgagcccaacttggtcagagatcgaggaggatttgagagcgtgcttcggtgcggaaccgttgaagaaagacttcagcgagccgctgaacttggactaa

SEQ ID NO: 14 - DNA, 2042 bp, Mouse parvovirus 4a
atggctggaaatgcttactctgatgaagttttgggagcaaccaactggttaaaggaaaaaaataatcaggaagtgttctcatttgtttttaaaaatgaggatgttcaactgaatggaaaagatatcggatggaatagttacaaaaaggagctgcaggaggacgagctgaaatctttacaacgaggagcggaaactacctgggaccaaagcgaggacatggaatgggaatctgcagtggatgaagtgaccaaaaagcaagtattcatttttgactctttagttaaaaaatgtttgtttgaagtgcttaacacaaagaacatagctcctgctgatgttaattggtttgtgcagcatgaatggggaaaagaccaaggctggcactgccatgtactaattggaggcaaggactttagtcaagctcaaggaaagtggtggagaaggcagctaaatgtttactggagcagatggttagtaacagcctgtaatgtacagctatcaccagctgaaagaattaaactaagagaaatagcagaagacaatgagtgggttaccttgctcacttataagcataagcaaaccaaaaaggactatactaagtgtgttctttttggcaacatgattgcttactactttttaaccaaaaagaaaataagcactagtccaccaagggacggaggctattttctgagcagtgactctggctggaaaactaactttttaaaagagggcgaacgccatctagtgagcaaactatatactgatgacatgcggccagaaacggttgaaaccacagtaaccactgcgcaggaaactaagcgcggcagaattcaaactaaaaaagaggtttcaattaaaaccacacttaaagagctggtgcataaaagagtaacctcaccagaagactggatgatgatgcagccagacagttacattgaaatgatggctcaaccaggtggagaaaacctgctgaaaaatacgctagagatttgtacactaactctagccagaaccaaaacagcatttgacttgattttagaaaaagctgaaaccagcaaactaacaaacttttcactgcctgatacaagaacctgcaagatttttgcttttcatggctggaactacattaaagtttgccatgctatttgctgtgttttaaacagacaaggaggcaaaagaaatactgttttatttcatggaccagccagtacaggcaaatctatcattgcacaagccatagcacaggcagttggtaatgttggttgctataatgcagcaaatgtgaactttccattcaatgactgtaccaacaagaacttaatttgggtggaagaagctggtaactttggacaacaagtaaaccagtttaaagccatttgctctggtcaaactattcgcattgatcaaaaaggaaaaggcagcaagcagattgaaccaacaccagtcatcatgaccacaaatgaaaacatcacagtggtcagaataggctgcgaagagagaccagaacacactcaaccaatcagagacagaatgcttaacattcatctaacacatacattgcctggtgactttggtttggttgacaaaaatgagtggcccatgatttgtgcttggttggtaaagaatggttaccaatctaccatggcaagctactgtgctaaatggggcaaagttcctgattggacagaaaactgggcggagccgaaggtgccgactcctataaattcactaggttcggcacgctcaccattcacgacaccgaaaagtacgcctctcagccagaactatgcactaactccacttgcatcggatctcgaggacctggctttagagccttggagcacaccaaatactcctgttgcgggcactgcagaaacccagaacactggggaagctggttccaaagcctgccaagatggtcaactgagcccaacttggtcagagatcgaggaggatttgagagcgtgcttcggtgcggaaccgttgaagaaagacttcaacgagccgctgaacttggactaaggtacgatggcgcctccagctaa

SEQ ID NO: 15 - DNA, 2019 bp, Mouse parvovirus 1b
atggctggaaatgcttactctgatgaagttttgggaacaaccaactggttaaaggaaaaaagtaaccaggaagtgttctcatttgtttttaaaactgaggatgttcaactaaatggaaaagatatcggatggaataattacaaaaaggagctgcaggaggacgagctgaaatctttacaacgaggagcggaaactacctgggaccaaagcgaggacatggaatgggaatctacagtggatgaaatgaccaaaaagcaagtattcatttatgactctttagttaaaaaatgtttgtttgaagtgcttagcacaaagaatatagctcctgctgatgttacttggtttgtgcagcatgaatgggggaaagaccaaggctggcactgccatgtactaattggaggcaaggactttagtcaagctcaaggaaaatggtggagaaggcagctaaatgtttactggagcagatggttggtaacagcctgtaatgtgcagctaacaccagctgaaagaattaaactaagagaaatagcagaagacagtgagtgggttactttgctcacttataagcataagcaaaccaaaaaggactataccaagtgtgttctttttggaaacatgattgcttactactttttaaccaagaagaaaataagcactagtccgccaagggacggaggctattttctgagcagtgactctggctggaaaactaactttttaaaagagggcgaacgccatctagtgagcaaactatacactgatgacatgcggccagaaacggttgaaaccacagtaaccactgcgcaggaaactaagcgcggcagaattcaaactaaaaaagaggtttctattaaaaccacacttaaagagctggtgcataaaagagtaacctcaccagaagactggatgatgatgcagccagacagttacattgaaatgatggctcaaccaggtggagaaaacctgctgaaaaatacgctagagatctgtacactaactctagctagaaccaaaacagcatttgacttgattttagaaaaagctgaaaccagcaaactaaccaacttttcactgcctgacacaagaacctgcaagatctttgcttttcatggctggaactacattaaagtttgccatgctatttgctgtgttctaaacagacaaggaggcaaaagaaatactgttttatttcatggaccagccagtacaggcaaatccattattgcacaagccatagcacaggcagttggtaatgttggttgctataatgcagcaaatgtgaactttccattcaatgactgtaccaacaagaacttgatttgggtggaagaagctggtaactttggacagcaagtaaaccagtttaaagccatttgctctggtcaaacaattcgcattgatcaaaaaggaaaaggcagcaagcagattgaaccaacaccagtcatcatgaccacaaatgagaacattacagtggtcaaaataggctgcgaggagagaccagaacacactcaaccaatcagagacagaatgcttaacattcatctaacacatacattgcctggtgactttggtttggttgacaaaagtgagtggcccatgatctgtgcttggttggtaaagaatggttaccaatctaccatggcaagctactgtgctaaatggggcaaagttcctgattggacagaaaactgggcggagccgaaggtgccgactcctataaattcactaggttcggcacgctcaccattcacgacaccgaaaagtacgcctctcagccagaactatgcactaactccacttgcatcggatctcgaggacctggctttagagccttggagcacaccaaatactcctgttgcgggcactgcagaaacccagaacactggggaagctggttccaaagcctgccaagatggtcaactgagcccaacttggtcagagatcgaggaggatttgagagcgtgcttcggtgcggaaccgttgaagagagacttcagcgagccgctgaacttggactaa

SEQ ID NO: 16 - DNA, 2019 bp, Mouse parvovirus minute virus immunosuppressive variant
atggctggaaatgcttactctgatgaagttttgggaacaaccaactggttaaaggaaaaaagtaaccaggaagtgttctcatttgtttttaaaactgaggatgttcaactaaatggaaaagatatcggatggaataattacaaaaaggagctgcaggaggacgagctgaaatctttacaacgaggagcggaaactacctgggaccaaagcgaggacatggaatgggaatctacagtggatgaaatgaccaaaaagcaagtattcatttatgactctttagttaaaaaatgtttgtttgaagtgcttagcacaaaaaatatagctcctgctgatgttacttggtttgtgcagcatgaatgggggaaagaccaaggctggcactgccatgtactaattggaggcaaggactttagtcaagctcaaggaaaatggtggagaaggcagctaaatgtttactggagcagatggttggtaacagcctgtaatgtgcagctaacaccagctgaaagaattaaactaagagaaatagcagaagacagtgagtgggttactttactcacttataaacataagcaaaccaaaaaggactatactaaatgtgttctttttggaaatatgattgcttactactttttaaccaaaaagaaaataagcaccagtccgccaagggacggaggctattttctaagcagtgactctggctggaaaactaactttttaaaagagggcgaacgccatctagtgagcaaattatacactgatgacatgcggccagaaacggttgaaaccacagtaaccactgcgcaggaaactaagcgcggcagaattcaaactaaaaaagaggtttctattaaaaccacacttaaagagctagtgcataaaagagtaacctcaccagaagactggatgatgatgcagccagacagttacattgaaatgatggctcaaccaggtggagaaaacctgctgaaaaatacgctagagatttgtacgctaactctagccagaacaaaaacagcatttgacttgattttagaaaaagctgaaaccagcaaactaaccaacttttcactgcctgacacaagaacctgcaagatttttgcttttcatggctggaactatgttaaagtttgccatgctatttgctgtgttctaaacagacaaggaggcaaaagaaatactgttttatttcacggaccagccagtacaggcaaatctattattgcacaagccatagcacaggcagttggtaatgttggttgctataatgcagctaatgtgaactttccatttaatgactgtacgaacaaaaacttgatttgggtagaagaagctggtaactttggacagcaagtaaaccagtttaaagccatttgctctggtcaaactattcgcattgatcaaaaaggaaaaggcagcaaacaaattgaaccaacaccagtcatcatgaccacaaatgagaacattacagtggtcagaataggctgcgaagagagaccagaacacactcaaccaattagagacagaatgctcaacattcatctaacacatacattgcctggtgactttggtttggttgacaagaatgaatggcccatgatttgtgcttggttggtaaagaatggttaccaatctaccatggcaagctactgcgctaaatggggcaaagttcctgattggtcagaaaactgggcggagccgaaggtgccgactcctataaattcactaggttcggcacgctcaccattcacgacaccgaaaagtacgcctctcagccagaactatgcactaactccacttgcatcggatctcgaggacctggctttagagccttggagcacaccaaatactcctgttgcgggcactgcagaaacccagaacactggggaagctggttccaaagcctgccaagatggtcaactgagcccaacttggtcagagatcgaggaggatttgagagcgtgcttcggtgcggaaccgttgaagagagacttcagcgagccgctgaacttggactaa

SEQ ID NO: 17 - DNA, 2019 bp, Mouse parvovirus 1
atggctggaaatgcttactctgatgaagttttgggaacaaccaactggttaaaggaaaaaagtaaccaggaagtgttctcatttgtttttaaaactgaggatgttcaactaaatggaaaagatatcggatggaataattacaaaaaggagctgcaggaggacgagctgaaatctttacaacgaggagcggaaactacctgggaccaaagcgaggacatggaatgggaatctacagtggatgaaatgaccaaaaagcaagtattcatttatgactctttagttaaaaaatgtttgtttgaagtgcttagcacaaagaatatagctcctgctgatgttacttggtttgtgcagcatgaatgggggaaagaccaaggctggcactgccatgtactaattggaggcaaggactttagtcaagctcaaggaaaatggtggagaaggcagctaaatgtttactggagcagatggttggtaacagcctgtaatgtgcagctaacaccagctgaaagaattaaactaagagaaatagcagaagacagtgagtgggttactttacttacttataaacataagcaaaccaaaaaggactatactaaatgtgttctttttggaaatatgattgcttactactttttaaccaaaaaaaaaataagcaccagtccgccaagagacggaggctattttctaagcagtgactctggctggaaaactaactttttaaaagaaggcgaacgccatctagtgagcaaactatacactgatgacatgcgaccagaaacggttgaaaccacagtaaccactgcgcaggaaactaagcgcggcagaattcaaactaaaaaagaggtttctattaaaaccacacttaaagagctggtgcataaaagagtaacctcaccagaagactggatgatgatgcagccagacagttacattgaaatgatggctcaaccaggtggagaaaacctgctgaaaaatacgctagagatctgtacactaactctagctagaaccaaaacagcatttgacttgattttagaaaaagctgaaaccagcaaactaaccaacttttcactgcctgacacaagaacctgcaagatctttgcttttcatggctggaactacattaaagtttgccatgctatttgctgtgttctaaacagacaaggaggcaaaagaaatactgttttatttcatggaccagccagtacaggcaaatccattattgcacaagccatagcacaggcagttggtaatgttggttgctataatgcagcaaatgtgaactttccattcaatgactgtaccaacaagaacttaatttgggtggaagaagctggtaactttggacaacaagtaaaccagtttaaagccatttgctctggtcaaacaattcgcattgatcaaaaaggaaaaggcagcaagcagattgaaccaacaccagtcatcatgaccacaaatgaaaacattacagtggtcaaaataggctgcgaggaaagaccagaacacactcaaccaatcagagacagaatgcttaacattcatctaacacatacattgcctggtgactttggtttggttgacaaaaatgagtggcccatgatttgtgcttggttggtaaagaatggttaccaatctaccatggcaagctactgtgctaaatggggcaaagttcctgattggacggaaaactgggcggagccgaaggtgccgactcctataaattcactaggttcggcacgctcaccattcacgacaccgaaaagtacgcctctcagccagaactatgcactaactccacttgcatcggatctcgaggacctggctttagagccttggagcacaccaaatactcctgttgcgggcactgcagaaacccagaacactggggaagctggttccaaagcctgccaagatggtcaactgagcccaacttggtcagagatcgaggaggatttgagagcgtgcttcggtgcggaaccgttgaagaaagacttcagcgagccgctgaacttggactaa

SEQ ID NO: 18 - DNA, 2019 bp, Mouse parvovirus 5a
atggctggaaatgcttactctgatgaagttttgggaacaaccaactggttaaaggaaaaaagtaaccaggaagtgttctcatttgtttttaaaactgaagatgttcaactgaatggaaaagatattggatggaataattacagaaaggagctgcaagaggacgagctaaaatctttacaacgaggagcggaaactacctgggaccaaagcgaggacatggaatgggaatctacagtggatgaagtgaccaaaaagcaagtattcatttatgactctttagttaaaaaatgtttgtttgaagtacttagcacaaagaacatagctcctagtgatgttaattggtttgtgcagcatgaatggggaagagaccaaggctggcattgccatgtactaattggaggcaaagactttagtcaagctcaaggaaagtggtggagaaggcagctaagtgtttactggagcagatggttggtaacagcttgtaatgtacagctaacaccagctgaaagaattaaactaagagaaatagcagaagacagtgaatgggttaccttgctcacttataagcataagcaaaccaaaaaggactataccaagtgtgttctttttggaaacataattgcttactactttttaactaaaaagaaaataagcaccagtccgccaagagacggaggctattttcttagcagtgactctggctggaaaactaactttttaaaagagggcgaacgccatctagtgagcaaactatacactgatgacatgcggccagaaacggttgaaaccacagtaaccactgcgcaggaaactaagcgcggcagaattcaaactaaaaaagaggtttcaattaaaaccacacttaaagagctggtgcataagagagtaacctcaccagaagactggatgatgatgcagccagacagttatattgaaatgatggctcaaccaggtggagaaaacctgctaaaaaatacgctagagatttgtacactaactctagctagaaccaaaacagcatttgacttgattttagaaaaagctgaaaccagcaaactaaccaacttttcactgccggacacaagaacctgcaaaatttttgcttttcatggctggaactatgttaaagtttgccatgctatttgctgtgttctaaacagacaaggaggcaagagaaatactgttttatttcatggaccagccagcacaggcaaatccattattgcacaagccatagcacaggcagttggtaatgttggttgctataatgcagcaaatgtgaactttccattcaatgactgtaccaacaagaacttaatttgggtggaagaagctggtaactttggacaacaagtaaaccagtttaaagccatttgctctggtcaaacaattcgcattgatcaaaaaggaaaaggcagcaagcagattgaaccaacaccagtcatcatgaccacaaatgaaaacattacagtggtcaaaataggctgcgaggaaagaccagaacacactcaaccaatcagagacagaatgcttaacattcatctaacacatacattgcctggtgactttggtttggttgacaaaaatgagtggcccatgatttgtgcttggttggtaaagaatggttaccaatctaccatggcaagctactgtgctaaatggggcaaagttcctgattggacggaaaactgggcggagccgaaggtgccgactcctataaattcactaggttcggcacgctcaccattcacgacaccgaaaagtacgcctctcagccagaactatgcactaactccacttgcatcggatctcgaggacctggctttagagccttggagcacaccaaatactcctgttgcgggcactgcagaaacccagaacactggggaagctggttccaaagcctgccaagatggtcaactgagcccaacttggtcagagatcgaggaggatttgagagcgtgcttcggtgcggaaccgttgaagaaagacttcagcgagccgctgaacttggactaa

SEQ ID NO: 19 - DNA, 2019 bp, Mouse parvovirus UT
atggctggaaacgcttactctgatgaagttttgggaacaaccaactggttaaaggaaaaaagtaaccaggaagtgttctcatttgtttttaaaactgaggatgttcaactaaatggaaaagatatcggatggaataattacagaaaggagctgcaggaggacgagctgaaatctttacaacgaggagcagaaactacctgggaccaaagcgaggacatggaatgggaatctacagtggatgaagtgaccaaaaagcaagtattcatttatgactctttagttaaaaaatgtttgtttgaagtgcttaacacaaagaacatatctcctggtgatgttaattggtttgtgcagcatgaatggggaaaagaccaaggctggcattgccatgtactaattggaggcaaagactttagccaagctcaaggaaagtggtggagaaggcagctaagtgtttactggagcagatggttagtaacagcctgtaatgtgcagctatcaccagctgaaagaattaaactaagagaaatagcagaagacagtgagtgggttaccttgctcacttataagcataagcaaaccaaaaaagactatactaagtgtgttctttttggcaacataattgcttactactttttaaccaagaagaaaataagcactagtccgccaagggacggaggctattttctgagcagtgactctggctggaaaactaactttttaaaagagggcgaacgccatctagtgagcaaactatacactgatgacatgcggccagaaacggttgaaaccacagtaaccactgcgcaggaaactaagcgcggcagaattcaaactaaaaaagaagtttctattaaaaccacacttaaagaactggtgcataaaagagtaacctcaccagaagactggatgatgatgcagccagacagttacattgaaatgatggctcaaccaggtggagaaaacctgctaaaaaatacgctagagatttgtacgctaactctagctagaaccaaaacagcatttgacttgattttagaaaaagctgaaaccagcaaactaactaacttttcactgcctgacacaagaacctgcaagatttttgcttttcatggctggaactacattaaagtttgccatgctatttgctgtgttctaaacagacaaggaggcaaaagaaatactgttttatttcatggaccagccagtacaggcaaatccattattgcacaagccatagcacaggcagttggtaatgttggttgctataatgcagcaaatgtgaactttccattcaatgactgtaccaacaagaacttgatttgggtggaagaagctggtaactttggacagcaagtaaaccagtttaaagccatttgctctggtcaaacaattcgcattgatcaaaaaggaaaaggcagcaagcagattgaaccaacaccagtcatcatgaccacaaatgagaacattacagtggtcaaaataggctgcgaggagagaccagaacacactcaaccaataagagacagaatgcttaacattcatctaacacatacattgcctggtgactttggtttggttgacaaaagtgagtggcccatgatctgtgcttggttggtaaagaatggttaccaatctaccatggcaagctactgtgctaaatggggcaaagttcctgattggtcagaaaactgggcggagccgaaggtgccgactcctataaattcactaggttcggcacgctcaccattcacgacaccgaaaagtacgcctctcagccagaactatgcactaactccacttgcatcggatctcgaggacctggctttagagccttggagcacaccaaatactcctgttgcgggcactgcagaaacccagaacactggggaagctggttccaaagcctgccaagatggtcaactgagcccaacttggtcagagatcgaggaggatttgagagcgtgcttcggtgcggaaccgttgaagaaagacttcagcgagccgctgaacttggactaa

SEQ ID NO: 20 - DNA, 2009 bp, Mouse parvovirus 1e
atgcttactctgatgaagttttgggaacaaccaactggttaaaggaaaaaagtaaccaggaagtgttctcatttgtttttaaaactgaagatattcaactgaatggaaaagatattggatggaataattacagaaaggagctgcaagaggacgagctaaaatctttacaacgaggagcggaaactacctgggaccaaagcgaggacatggaatgggaatctacagtggatgaagtgaccaaaaagcaagtattcatttatgactctttagttaaaaaatgtttgtttgaagtgcttaacacaaagaacatatctcctggtgatgttaattggtttgtgcagcatgaatggggaagagaccaaggctggcattgccatgtactaattggaggcaaagactttagtcaagctcaaggaaagtggtggagaaggcagctaagtgtttactggagcagatggttggtaacagcctgtaatgtacagctaacaccagctgaaagaattaaactaagagaaatagcagaagacagtgaatgggttaccttgctcacttataagcataagcaaaccaaaaaggactataccaagtgtgttctttttggcaacataattgcttactactttttaaccaagaagaaaataagcaccagtccgccaagggacggaggctattttcttagtagtgactctggctggaaaactaactttttaaaagagggcgaacgccatctagtgagcaaactatacactgatgacatgcggccagaaacggttgaaaccacagtaaccactgcgcaggaaactaagcgcggcagaattcaaactaaaaaagaggtttctattaaaaccacacttaaagagctagtgcataagagagtaacctcaccagaagactggatgatgatgcagccagacagttatattgaaatgatggctcaaccaggtggagaaaacctgctgaaaaatacgctagagatctgtacactaactctagctagaaccaaaacagcatttgacttgattttagaaaaagctgaaaccagcaaactaaccaacttttcactgcctgacacaagaacctgcaagatctttgcttttcatggctggaactacattaaagtttgccatgctatttgctgtgttctaaacagacaaggaggcaaaagaaatactgttttatttcatggaccagccagtacaggcaaatccattattgcacaagccatagcacaggcagttggtaatgttggttgctataatgcagcaaatgtgaactttccattcaatgactgtaccaacaagaacttaatttgggtggaagaagctggtaactttggacaacaagtaaaccagtttaaagccatttgctctggtcaaacaattcgcattgatcaaaaaggaaaaggcagcaagcagattgaaccaacaccagtcatcatgaccacaaatgaaaacattacagtggtcaaaataggctgcgaggaaagaccagaacacactcaaccaatcagagacagaatgcttaacattcatctaacacatacattgcctggtgactttggtttggttgacaaaaatgagtggcccatgatttgtgcttggttggtaaagaatggttaccaatctaccatggcaagctactgtgctaaatggggcaaagttcctgattggacggaaaactgggcggagccgaaggtgccgactcctataaattcactaggttcggcacgctcaccattcacgacaccgaaaagtacgcctctcagccagaactatgcactaactccacttgcatcggatctcgaggacctggctttagagccttggagcacaccaaatactcctgttgcgggcactgcagaaacccagaacactggggaagctggttccaaagcctgccaagatggtcaactgagcccaacttggtcagagatcgaggaggatttgagagcgtgcttcggtgcggaaccgttgaagagagacttcagcgagccgctgaacttggactaa

SEQ ID NO: 21 - DNA, 2019 bp, Mouse parvovirus 1c
  misc_feature (609)..(609): n is a, c, g, or t
  misc_feature (1590)..(1590): n is a, c, g, or t
atggctggaaatgcttactctgatgaagttttgggaacaaccaactggttaaaggaaaaaagtaaccaggaagtgttctcatttgtttttaaaactgaagatgttcaactaaatggaaaagatattggatggaataattacagaaaggagctgcaagaggacgagctaaaatctttacaacgaggagcggaaactacctgggaccaaagcgaggacatggaatgggaatctacagtggatgaagtgaccaaaaagcaagtattcatttatgactctttagttaaaaaatgtttgtttgaagtgcttaacacaaagaacatatctcctggtgatgttaattggtttgtgcagcatgaatggggaagagaccaaggctggcattgccatgtactaattggaggcaaagactttagtcaagctcaaggaaagtggtggagaaggcagctaagtgtttactggagcagatggttggtaacagcctgtaatgtacagctaacaccagctgaaagaattaaactaagagaaatagcagaagacagtgaatgggttaccttgctcacttataagcataagcaaaccaaaaaggactataccaagtgtgttcttttnggcaacataattgcttactactttttaaccaagaagaaaataagcaccagtccgccaagggacggaggctattttcttagtagtgactctggctggaaaactaactttttaaaagagggcgaacgccatctagtgagcaaactatacactgatgacatgcggccagaaacggttgaaaccacagtaaccactgcgcaggaaactaagcgcggcagaattcaaactaaaaaagaggtttctattaaaaccacacttaaagagctagtgcataagagagtaacctcaccagaagactggatgatgatgcagccagacagttatattgaaatgatggctcaaccaggtggagaaaacctgctgaaaaatacgctagagatctgtacactaactctagctagaaccaaaacagcatttgacttgattttagaaaaagctgaaaccagcaaactaaccaacttttcactgcctgacacaagaacctgcaagatctttgcttttcatggctggaactacattaaagtttgccatgctatttgctgtgttctaaacagacaaggaggcaaaagaaatactgttttatttcatggaccagccagtacaggcaaatccattattgcacaagccatagcacaggcagttggtaatgttggttgttataatgcagcaaatgtgaactttccattcaatgactgtaccaacaagaacttaatttgggtggaagaagctggtaactttggacaacaagtaaaccagtttaaagccatttgctctggtcaaacaattcgcattgatcaaaaaggaaaaggcagcaagcagattgaaccaacaccagtcatcatgaccacaaatgaaaacattacagtggtcaaaataggctgcgaggaaagaccagaacacactcaaccaatcagagacagaatgcttaacattcatctaacacatacattgcctggtgactttggtttggttgacaaacatgantggcccatgatttgtgcttggttggtaaagaatggttaccaatctaccatggcaagctactgtgctaaatggggcaaagttcctgattggacggaaaactgggcggagccgaaggtgccgactcctataaattcactaggttcggcacgctcaccattcacgacaccgaaaagtacgcctctcagccagaactatgcactaactccacttgcatcggatctcgaggacctggctttagagccttggagcacaccaaatactcctgttgcgggcactgcagaaacccagaacactggggaagctggttccaaagcctgccaagatggtcaactgagcccaacttggtcagagatcgaggaggatttgaaagcgtgcttcggtgcggaaccgttgaagagagacttcagcgagccgctgaacttggactaa

SEQ ID NO: 22 - DNA, 2019 bp, Hamster parvovirus
atggctggaaatgcttactctgatgaagttttgggaacaaccaactggttaaaagagaaaagtaaccaggaagtgttctcatttgtttttaaaaatgaagatgttcagctcaatggaaaagatatcggatggaatagttacaaaaaggagctgcaagaggaagagctgaaatctttacaacgaggagcggaaactacctgggaccagagcgaggacatggaatgggaatcttcagtggatgaactaaccaaaaagcaagtattcatttttgactctttagttaaaaaatgtttgtttgaagtgctgagtacaaagaacatagcacctagtgatgttacttggtttgtacagcatgaatggggaaaagaccaaggctggcactgtcatgtactaattggaggcaaggactttagccaagctcaaggaaaatggtggagaaggcagttaaatgtttactggagcagatggttggtaacagcctgtagtgtgcagctattaccagctgaaagaattaagctgagagagatagcggaagaccaagaatgggtcactttgcttacttataagcataagcaaaccaaaaaagactataccaagtgtgtttgctttggaaatatagttgcttactactttttatccaagaagaaaatatgcaccagtccaccaagggacggaggctattttcttagcagtgactctggctggaaaactaactttttaaaagaaggcgaacgccatctagtgagcaaactatacactgatgacatgcggccagaaacggttgaaaccacagtaaccactgcgcaggaaactaagcgcggcagaattcaaactaaaaaagaggtctctattaaaaccacacttaaagagctggtgcataagagagtaacctcaccagaagactggatgatgatgcagccagacagttacattgaaatgatggctcaaccaggtggagaaaacctgctgaaaaatacgctagagatttgtacactaactctagccagaacaaaaacagcatttgacttaattttagaaaaagctgaaaccagcaaactaaccaacttttcactgccggacacaagaacctgcaagatctttgcttttcatggctggaactatattaaagtttgccatgctatttgctgtgttctaaacagacaaggaggcaaaagaaatactgttttatttcatggaccagccagtacaggcaaatccattattgcacaagccatagcacaggcagttggtaatgttggttgctataatgcagcaaatgtgaactttccatttaatgactgcaccaacaaaaacctgatttgggtggaagaagctggtaactttggacagcaagtaaaccagtttaaagccatttgctctggtcaaactattcgcattgatcaaaaaggaaaaggcagcaaacagattgaaccaacaccagtcatcatgaccacaaatgaaaacattacagtggtcaaaataggctgtgaagaaagaccagaacacactcaaccaatcagagacagaatgcttaacattcatctaacacatacattgcctggtgactttggtttggttgacaaacatgaatggcccatgatttgtgcttggttggtaaagaatggttaccaatctaccatggcaagctactgtgctaaatggggcaaagttcctgattggacggaaaactgggcggagccgaaggtgccgactcctataaattcactaggttcggcacgctcaccattcacgacaccgaaaagtacgcctctcagccagaactatgcactaactccacttgcatcggatctcgaggacctggctttagagccttggagcacaccaaatactcctgttgcgggcactgcagaaacccagaacactggggaagctggttccaaagcctgccaagatggtcaactgagcccaacttggtcagagatcgaggaggatttgagagcgtgcttcggtgcggaaccgttgaagagagacttcagcgagccgctgaacttggactaa

SEQ ID NO: 23 - DNA, 2019 bp, Mouse parvovirus 3
atggctggaaacgcttactctgatgaagttttaggaacaaccaactggttaaaggaaaaaagtaaccaggaagtgttctcatttgtttttaaaaatgaagatgttcaactgaatggaaaagatatcggatggaataattacagaaaggagctgcaggaggacgagctgaaatctttacaacgaggagcggaaactacctgggaccaaagcgaggacatggaatgggaatctgcagtggatgaactaaccaaaaagcaagtattcatttatgactctttagttaaaaaatgtttgtttgaagtgctgagtacaaagaacatagctcctagtgatgttacttggtttgtacggcatgaatggggaaaagaccaaggctggcactgtcatgtgctcattggaggcaaggactttagccaagctcaaggaaaatggtggagaaggcagttaaatgtttactggagcagatggttagtaacagcctgtaatgtgcagttatcaccagctgaaagaattaagctgagagagatagcggaagaccaagaatgggtcactttgcttacttataagcataagcaaaccaaaaaggactataccaagtgtgttctttttggaaatatagttgcttactactttttaaccaagaagaaaataagcaccagtccaccaagggacggagactattttctgagcagtgactctggctggaaaactaactttttaaaagagggcgaacgccatctagtgagcaaactatacactgatgacatgcgaccagaaacggttgaaaccacagtaaccactgcgcaggaaactaagcgcggcagaattcaaactaagaaagaggtctctattaaaaccacacttaaagagctggtgcataaaagagtaacctcaccagaagactggatgatgatgcagccagacagttacattgaaatgatggctcaaccaggtggagaaaacctgctgaaaaatacgctagagatttgtacactaactctagccagaacaaaaacagcatttgacttgattttagaaaaagctgaaaccagcaaactaaccaacttttcactgccggacacaagaacctgcaagatctttgcttttcatggctggaactatattaaagtttgccatgctatttgctgtgttctaaacagacaaggaggcaaaagaaatactgttttatttcatggaccagccagtacaggcaaatccattattgcacaagccatagcacaggcagttggtaatgttggttgctataatgcagcaaatgtgaactttccattcaatgactgcaccaacaaaaacctgatttgggtagaagaagctggtaactttggacagcaagtaaaccaatttaaagccatttgctctggtcaaactattcgcattgatcaaaaaggaaaaggcagcaaacagattgaaccaacaccagtcatcatgaccacaaatgaaaacattacagtggtcaaaataggctgtgaagaaagaccagaacacactcaaccaatcagagatagaatgcttaacattcatctaacacatacattgcctggtgactttggtttggttgacaaacatgaatggcccatgatttgtgcttggttggtaaagaatggttaccaatctaccatggcaagctactgtgctaaatggggcaaagttcctgattggacggaaaactgggcggagccgaaggtgccgactcctataaattcactaggttcggcacgctcaccattcacgacaccgaaaagtacgcctctcagccagaactatgcactaactccacttgcatcggatctcgaggacctggctttagagccttggagcacaccaaatactcctgttgcgggcactgcagaaacccagaacactggggaagctggttccaaagcctgccaagatggtcaactgagcccaacttggtcagagatcgaggaggatttgagagcgtgcttcggtgcggaaccgttgaagagagacttcagcgagccgctgaacttggactaa

SEQ ID NO: 24 - DNA, 2019 bp, Mouse minute virus
atggctggaaatgcttactctgatgaggttttgggagcaaccaactggttaaaggaaaaaagtaaccagttagtattctcatttgtttttaaaaatgaagatgttcaattgaatggaaaagatatcggatggaatagttacagaaaggagctgcaagaggacgagctaaaatctttacaacgaggagcggaaactacctgggaccagagcgaggacatggaatgggaatcttcagtggatgaactaaccacaaagcaagtattcatttttgactctttagttaaaaagtgtttatttgaagtgctaagtacaaagaacatagctcctagtgatgttaattggtatgtgcagcatgaatggggaaaagaccaaggctggcattgccatgtactaattggaggcaaagactttagccaagctcaaggaaagtggtggagaaggcagctaaatgtttactggagcagatggttggtaacagcctgcagtgtgcagctatcaccagccgaaagaattaagctgagagaaatagcggaagaccaagaatgggtcactttgcttacttataagcataagcaaaccaaaaaagactataccaaatgtgtttgctttggaaatatgattgcttactactttttaaccaagaagaaaatatgcactagtccaccaagggacggaggctattttcttagcagtgactctggctggaaaactaactttttaaaagaaggcgaacgccatctagtgagcaaactatacactgatgacatgcggccagaaacggttgaaaccacagtaaccactgcgcaggaaactaagcgcggcagaattcaaactaaaaaagaggtttctattaaaaccacacttaaagagctggtgcataagagagtaacctcaccagaagactggatgatgatgcagccagacagttacattgaaatgatggctcagccaggtggagaaaacctgcttaaaaatacgctagagatctgtacgctaactctagctagaaccaaaacagcctttgacttgattttagaaaaagctgaaaccagcaaactaaccaacttttcactgccggacacaagaacctgtaagatttttgcttttcatggctggaactacattaaagtttgccatgctatttgctgtgttctaaacagacaaggaggcaaaagaaatactgttttatttcatggaccagccagtacaggcaaatccatcattgcacaagccatagcacaggcagttggtaatgttggttgctataatgcagcaaatgtgaactttccattcaatgactgcaccaacaaaaacctgatttgggtggaagaagctggtaactttggacagcaagtaaaccaatttaaagccatttgctctggtcaaactattcgcattgatcaaaaaggaaaaggcagcaagcagattgaaccaacaccagtcatcatgaccacaaatgagaacattacagtggtcagaataggctgcgaagagagaccagaacacactcaaccaattagagacagaatgctcaacattcatctaacacatacattgcctggtgactttggtttggttgacaaaaatgaatggcccatgatttgtgcttggttggtaaagaatggttaccaatctaccatggcaagctactgtgctaaatggggcaaagttcctgattggtcagaaaactgggcggagccgaaggtgccgactcctataaattcactaggttcggcacgctcaccattcacgacaccgaaaagtacgcctctcagccagaactatgcactaactccacttgcatcggatctcgaggacctggctttagagccttggagcacaccaaatactcctgttgcgggcactgcagaaacccagaacactggggaagctggttccaaagcctgccaagatggtcaactgagcccaacttggtcagagatcgaggaggatttgagagcgtgcttcggtgcggaaccgttgaagaaagacttcagcgagccgctgaacttggactaa

SEQ ID NO: 25 - DNA, 2019 bp, MVM strain M
atggctggaaatgcttactctgatgaagttttgggaacaaccaactggttaaaagagaaaagtaaccaggaagtgttctcatttgtttttaaaaatgaagatgttcagctcaatggaaaagatatcggatggaatagttacaaaaaggagctgcaagaggaagagctgaaatctttacaacgaggagcggaaactacctgggaccagagcgaggacatggaatgggaatcttcagtggatgaactaaccaaaaagcaagtattcatttttgactctttagttaaaaaatgtttgtttgaagtgctgagtacaaagaacatagctcctagtgatgttacttggtttgtacagcatgaatggggaaaagaccaaagctggcactgtcatgtactaattggaggcaaggactttagccaagctcaaggaaaatggtggagaaggcagttaaatgtttactggagcagatggttggtaacagcctgtagtgtgcagctatcaccagctgaaagaattaagctgagagagatagcggaagaccaagaatgggtcactttgcttacttataagcataagcaaaccaaaaaagactataccaagtgtgtttgctttggaaatatagttgcttactactttttatccaagaagaaaatatgcaccagtccaccaagggacggaggctattttcttagcagtgactctggctggaaaactaactttttaaaagaaggcgaacgccatctagtgagcaaactatacactgatgacatgcggccagaaacggttgaaaccacaataaccactgcgcaggaaactaagcgcggcagaattcaaactaaaaaagaggtctctattaaaaccacacttaaagagctggtacataagagagtaacctcaccagaagactggatgatgatgcagccagacagttacattgaaatgatggctcaaccaggtggagaaaacctgcttaaaaatacgctagaaatctgtacgctaactctagctagaaccaaaacagcatttgacttgattttagaaaaagctgaaaccagcaaactaaccaacttttcactgccggacacaagaacctgcaagatctttgcttttcatggctggaactatgttaaagtttgccatgctatttgctgtgttctaaacagacaaggaggcaaaagaaatactgttttatttcatggaccagccagtacaggcaaatccattattgcacaagccatagcacaggcagttggtaatgttggttgctataatgcagcaaatgtgaactttccatttaatgactgcaccaacaaaaacctgatttgggtggaagaagctggtaactttggacagcaagtaaaccagtttaaagccatttgctctggtcaaactatccgcattgatcaaaaaggaaaaggcagcaagcagattgaaccaacaccagtcatcatgaccacaaatgaaaacattacagtggtcagaataggctgcgaggagagaccagagcacactcaaccaatcagagacagaatgctcaacattcatctgacacatacattgcctggtgactttggtttggttgacaagaatgaatggcccatgatttgtgcttggttggtaaagaatggttaccaatctaccatggcaagctactgtgctaaatggggcaaagtacctgattggtcagaaaactgggcagagccgaaggtaccgactcctataaattcactaggttcagcacgctcaccattcacgacaccgaaaagtacgcctctcagccagaactatgcactaactccacttgcatcggatctcgaggacctggctttagagccttggagcacaccaaatactcctgttgcgggcactgcagaaacccagaacactggggaagctggttccaaagcctgccaagatggtcaactgagcccaacttggtcagagatcgaggaggatttgagagcgtgcttcggtgcggaaccgttgaagaaagacttcagcgagccgctgaacttggactaa

SEQ ID NO: 26 - DNA, 1966 bp, Parvovirus LuII
atggctggaaacgcgtactctgatgaagttttgggaacaactaactggttgaaggataagagcaaccaggaagtattctcatttgtttttaaaaatgaggatgttcagctcaatggaaaaaatatcggatggaacagttacagaaaggagctgcaagaggaggagctgaaatctttacaacgaggagctgaaactacctgggaccagagcgaggacatggaatgggaatcttcagtggatgaactgaccaaaaagcaagtattcatttttgactctttagttaaaaagtgtctctttgaagtactgagcacaaagaacatagctcctagtgatgttacttggtttgtacagcatgaatggggaaaagaccaaggctggcactgtcatgtgctcattggaggcaagaactttagccaggctcaaggaaaatggtggaggagacaattaaatgtttactggagtagatggttggtaacagcctgtagcgtgcagctatcaccagctgaaagaattaaactaagagaaatagcagaagaccaagaatgggttactctgcttacttataagcataagcaaaccaaaaaagactatactaagtgtgtttgctttggaaatatggttgcttactactttttaaccaaaaagaaaatatgtaccagtccaccaagggacggaggctattttctcagtagtgactctggctggaaaactaactttttgaaagaaggcgaacgccatctagtgagcaaactatatactgatgacatgcggccagaaacggttgagaccacagtaaccacagcgcaggaaactaagcgcggcagaattcaaactaagaaggaagtctctattaagactacacttaaagagctggtacataagagagtaacctcaccagaagactggatgatgatgcagccagacagttacattgaaatgatggctcaaccagggggagaaaacctacttaagaatacgctagagatctgtacgctgactctagccagaaccaaaacagcctttgacttgattttagaaaaagctgaaaccagcaaactaaccaactttttactggctgatacaagaacctgtagaatctttgcttttcatggctggaactacatcaaagtctgtcatgctatttgttgtgtcttgaacagacagggaggcaaaagaaatactgttctgtttcatggaccagccagtacaggcaaatcaatcattgcacaggccatagcacaggcagttggtaatgttggttgttataacgcagccaatgtgaactttccatttaatgactgtaccaacaagaacttaatctgggtggaagaagctggtaactttggacagcaagtaaaccagtttaaagccatttgttctggtcagaccattcgcattgaccaaaaaggaaaaggcagcaaacagattgaaccaacaccagtgatcatgaccacaaatgaaaacatcacagtggtcaaaatagggtgtgaagagagaccagaacacactcaaccaatcagagacagaatgttaaacattcatctgacacatacattgcctggtgactttggtttggttgataaaaacgaatggcctatgatatgtgcttggttggtaaagaacggttaccaatcgaccatggcaagttactgtgctaaatggggcaaagttcctgattggacagaaaactgggcggagccaaaagtaacgactgaaataaattcggtaggttcaaccaactcaccatctccgaaaagtacgcctctcagccagaactacgcactaactccgtcggatctcgaggacctggctctggagccttggagcacaccaagtactcctgttgtgggcactgtcaaaaccccgaacactggggaaactggttcaacagcctgtcaagaagctcaacggagcccaacttggtccgagatcgaggaggatttgagagcgtgcttcagttcggaac

SEQ ID NO: 27 - DNA, 2019 bp, Rat parvovirus UT
atggctggaaacgcttactccgatgaggttttgggagcaaccaactggctaaaggacaaaagtagccaagaggtgttctcatttgtttttaaaaatgagaacgtccagctaaatgggaaggacatcggttggaatagttacagaaaggagctacaagatgacgagctgaagtctctacaacgaggagcggaaaccacttgggaccaaagcgaggacatggaatgggagagcgcagtggatgacatgaccaaaaagcaagtattcatttttgattctttggttaagaaatgtttgtttgaagtgctcagcacaaagaacataactcctagtgatgttacttggttcgtgcagcatgaatggggaaaggaccaaggctggcactgtcatgtgctaattggaggcaaagactttagtcaagctcaaggaaaatggtggagaaggcagctaaatgtgtactggagtagatggttggtgactgcctgtaatgttcaactaacaccagctgaaagaataaaactgagagaaatagcagaggacagtgaatgggtcactttgcttacctataagcataagcacaccaagaaggactataccaagtgtgttctttttggaaacatgattgcttattactttttaagcaaaaagaaaatatgtaccagtccaccaagggacggaggctattttcttagcagtgactctggctggaaaactaactttttgaaagagggcgagcgccatctagtgagcaagctgtatactgatgagatgaaaccagaaacggttgagaccacagtgaccacagcacaggaagctaagcgcggcagaattcaaactagaaaggaggtctctattaaaaccacacttaaagagttggtacataaaagagtaacctcaccagaagactggatgatgatgcagccagacagttacattgaaatgatggctcaaccaggtggagaaaacttgcttaaaaatacactagagatctgtacactgactctagcaagaaccaaaacagcatttgacttgattctggaaaaagctgaaaccagcaaactagccaacttttccatggctaacaccagaacctgtagaatctttgctgaacatggctggaactatattaaagtctgtcatgccatctgttgtgtgctaaatagacaaggaggcaaaaggaacactgtgctctttcatggaccagccagcacaggcaaatctattattgcacaagccatagcacaagcagttggtaatgttggttgttataatgctgccaatgtgaactttccatttaatgactgcaccaacaaaaacttgatttgggtggaagaagctggtaactttggccagcaagtaaaccaattcaaagctatttgttctggccaaaccatacgcattgatcaaaaaggaaaaggcagcaaacagattgaaccaacaccagttatcatgaccaccaacgagaacattaccgtggtcagaataggctgtgaggaaagaccagaacacactcaaccaatcagagacagaatgctcaacattcacctgacacgtacactgcctggtgactttggtctggtggataagcacgaatggcctctgatctgtgcttggttggtgaagaatggttaccaatctaccatggcttgttactgtgctaaatggggcaaagttcctgattggtcagaagactgggcggagccgaagctagagactcctataaattcactaggttcaatgcgctcaccatctctgactccgagaagtacgcctctcagccagaactacgctcttactccacttgcatcggaccttgcggacctagctctagagccttggagcacaccaaatactcctgttgtgggcactgcagcaagccagaacactggggaggctggtttcacagcctgccaaggtgctcaacggagcccaacctggtccgagatcgaggcggatctgagagcgtgcttcagccaggaacagctggagaaagacttcagcgattcactgaccttggactaa

SEQ ID NO: 28 - DNA, 2019 bp, Kilham rat virus
atggctggaaacgcttactccgatgaggttttgggagcaaccaactggctaaaggacaaaagtagccaggaggtgttctcatttgtttttaaaaatgagaacgtccaactaaatgggaaggacatcggttggaatagttacagaaaggagctacaagatgacgagctgaagtctctacaacgaggggcggagaccacttgggaccaaagcgaggacatggaatgggagagcgcagtggatgacatgaccaaaaagcaagtattcatttttgattctttggttaagaagtgtttgtttgaagtgctcagcacaaagaacatagctcctagtgatgttacttggttcgtgcagcatgaatggggaaaggaccaaggctggcactgtcatgtgctgattggaggcaaggactttagtcaagctcaaggaaaatggtggagaaggcagctaaatgtgtactggagtagatggttggtgactgcctgtaatgttcaactaacaccagctgaaagaattaaactgagagaaatagcagaagacagtgaatgggtcactttgcttacctataagcataagcacaccaagaaggactataccaagtgtgttctttttggaaacatgattgcttattactttctaagcaaaaagaaaatatgtaccagtccaccaagggacggaggctattttcttagcagtgactctggctggaaaactaactttttgaaagagggcgagcgccatctagtgagcaaactatatactgatgagatgaaaccagaaacggtcgagaccacagtgaccactgcgcaggaagctaagcgcggcagaattcaaactagaaaggaggtctcgattaaaaccacactcaaagagttggtgcataaaagagtaacctcaccagaagactggatgatgatgcagccagacagttacattgaaatgatggctcaaccaggtggagaaaacttgcttaaaaatacactagagatctgtacactgactctagcaagaaccaaaacagcctttgacttgattctggaaaaagctgaaaccagcaaactagccaacttttccatggctagcaccagaacctgtagaatctttgctgagcatggctggaactatattaaagtctgccatgccatctgttgtgtgctaaatagacaaggaggcaaaaggaacactgtgctctttcacggaccagccagcacaggcaaatctatcattgcacaagccatagcacaaggagttggtaatgttggttgttataatgctgccaatgtgaactttccatttaatgactgtaccaacaaaaacttgatttgggtggaagaagctggtaactttggccagcaagtaaaccaattcaaagctatttgttctggccaaaccatacgcattgatcaaaaaggaaaaggcagcaaacagattgaaccaacaccagttatcatgaccaccaacgagaacattaccgtggtcagaataggctgtgaggaaagaccagaacacactcaaccaatcagagacagaatgctcaacattcacctgacacgtacactgcctggtgactttggtctggtggataagcacgaatggcctctgatctgtgcttggttggtgaagaatggttaccaatctaccatggcttgttactgtgctaaatggggcaaagttcctgattggtcagaggactgggcggagccgaagctagagactcctataatttcgctaggttcaatgcgctcaccatctctgactccgagaagtacgcctctcagccagaactacgctcttactccacttgcatcggaccttgcggacctagctctagagccttggagcacaccaaatactcctgttgcgggcactgcagcaagccagaacactggggaggctggtttcacagcctgccaaggtgctcaacggagcccaacctggtccgagatcgaggcggatctgagagcgtgcttcagccaggaacagctggagaaagacttcagcgattcactgacattggactaa

SEQ ID NO: 29 - DNA, 2024 bp, Rat minute virus 1c
atggctggaaacgcttactccgatgaagttttgggagcaaccaactggctaaaggacaaaagtagccaggaagtgttctcatttgtttttaaaaatgagaacgtccaactaaatgggaaggacatcggttggaatagttacagaaaagagctacaagatgacgagctgaagtctctacaacgaggggcggagaccacttgggaccaaagcgaggacatggaatgggagagcgcagtggatgacatgaccaaaaagcaagtattcatttttgattctttggttaagaagtgtctgtttgaagtgctcagcacaaagaacatagctcctagtgatgttacttggttcgtgcagcatgaatggggaaaggaccaaggctggcactgtcatgtgctgattggaggcaaggactttagtcaagctcaaggaaaatggtggagaaggcagctaaatgtgtactggagtagatggttagtgactgcctgtaatgttcaactaacaccagctgaaagaattaaactgagagaaatagcagaggacagtgaatgggtcactttgcttacctataagcataagcacaccaagaaggactataccaagtgtgttctttttggaaacatgattgcttattactttctaagcaaaaagaaaatatgtaccagtccaccaagggacggaggctattttcttagcagtgactctggctggaaaactaactttttgaaagagggcgagcgccatctagtgagcaaactgtatactgatgagatgaaaccagaaacggtcgagaccacagtgaccactgcgcaggaagctaagcgcggcagaattcaaactagaaaggaggtctcgattaaaaccacactcaaagagttggtacataaaagagtaacctcaccagaagactggatgatgatgcagccagacagttacattgaaatgatggctcaaccaggtggagaaaacttgcttaaaaatacactagagatttgtacactgactctagcaagaaccaaaacagcctttgacttgattctggaaaaagctgaaaccagcaaactagccaacttttccatggctagcaccagaacctgtagaatctttgctgagcatggctggaactatattaaagtctgccatgccatctgttgtgtactaaatagacaaggaggcaaaaggaacactgtgctctttcacggaccagccagcacaggcaaatctatcattgcacaagccatagcacaaggagttggtaatgttggttgttacaatgctgccaatgtgaactttccatttaatgactgtaccaacaaaaacttgatttgggtggaagaagctggtaactttggccagcaagtaaaccaattcaaagctatttgttctggccaaaccatacgcattgatcaaaaaggaaaaggcagcaaacagattgaaccaacaccagttatcatgaccaccaacgagaacattacagtggtcagaataggctgtgaggaaagaccagaacacactcaaccaatcagagacagaatgctcaacattcacctgacacgtacactgcctggtgactttggtctggtggataagcacgaatggcctctaatctgtgcttggttggtgaagaatggttaccaatctaccatggcttgttactgtgctaaatggggcaaagttcctgattggtcagaggactgggcggagccgaagctagagactcctataaattcgctaggttcaatgcgctcaccatctctgactccgagaagtacgcctctcagccagaactacgctcttactccacttgcatcggaccttgcggacctagccctagagccttggagcacaccaaatactcctgttgcgggcactgcagcaagccagaacactggggaggctggtttcacagcctgtcaaggtgctcaacggagcccaacctggtccgagatcgaggcggatctgagagcgtgcttcagccaggaacagctggagaaagacttcagcgattcactgaccttggactaaggtac

SEQ ID NO: 30 - DNA, 2019 bp, Rat minute virus 1b
atggctggaaacgcttactccgatgaggttttgggagcaaccaactggctaaaggacaaaagtagccaggaggtgttctcatttgtttttaaaaatgagaacgtccaactaaatgggaaggacatcggttggaatagttacagaaaggagctacaagatgacgagctgaagtctctgcaacgaggggcggagaccacttgggaccaaagcgaggacatggaatgggagagcgcagtggatgacatgaccaaaaagcaagtattcatttttgattctttggttaagaagtgtctgtttgaagtgctcagcacaaagaacatagctcctagtgatgttacttggtttgtgcagcatgaatggggaaaagaccaaggctggcactgtcatgtgctgattggaggcaaggactttagtcaagctcaaggaaaatggtggagaaggcagctaaatgtgtactggagtagatggttggtgactgcctgtaatgttcaactaacaccagctgaaagaattaaactgagagaaatagcagaggacagtgaatgggtgactttgcttacctataagcataagcacaccaagaaggactataccaagtgtgttctttttggaaacatgattgcttattactttctaagcaaaaagaaaatatgtaccagtccaccaagggacggaggctattttcttagcagtgactctggctggaaaactaactttttgaaagagggcgagcgccatctagtgagcaaactgtatactgatgagatgaaaccagaaacggtcgagaccacagtgaccactgcgcaggaagctaagcgcggcagaattcaaactagaaaggaggtctcgattaaaaccacactcaaagagttggtgcataaaagagtaacctcaccagaagactggatgatgatgcagccagacagttacattgaaatgatggctcaaccaggtggagaaaacttgcttaaaaatacactagagatctgtacactgactctagcaagaaccaaaacagcctttgacttgattctggaaaaagctgaaaccagcaaactagccaactttttcatggctaacaccagaacctgtagaatctttgctgagcatggctggaactatattaaagtctgtcatgccatctgttgtgtgctaaatagacaaggaggcaaaaggaacactgtgctctttcacggaccagccagcacaggcaaatctatcattgcacaagccatagcacaaggagttggtaatgttggttgttataatgctgccaatgtgaactttccatttaatgactgtaccaacaaaaacttgatttgggtggaagaagctggtaactttggccagcaagtaaaccaattcaaagctatttgttctggccaaaccatacgcattgatcaaaaaggaaaaggcagcaaacagattgaaccaacaccagttatcatgaccaccaacgagaacattaccgtggtcaaaataggctgtgaggaaagaccagaacacactcaaccaatcagagacagaatgctcaacattcacctgacacgtacactgcctggtgactttggtctggtggataagcacgaatggcctctgatctgtgcttggttggtaaagaatggttaccaatctaccatggcttgttactgtgctaaatggggcaaagttcctgattggtcagaggactgggcggagccgaagctagagactcctataaattcgctaggttcaatgcgctcaccatctctgactccgagaagtacgcctctcagccagaactacgctcttactccacttgcatcggatctcgcggacctggcactggaaccttggagcacaccaaatactcctgttgtggacactgtacaaaccccgaacactggggaggctggtttcacagcctgccaaggtgctcaacggagcccaacctggtccgagatcgaggcggatctgagagcgtgcttcagccaggaacagctggagaaagacttcagcgattcactgaccttggactaa

SEQ ID NO: 31 - DNA, 1997 bp, Rat minute virus 1a
atgaggttttgggagcaaccaactggctaaaggacaaaagtagccaggaggtgttctcatttgtttttaaaaatgagaacgtccaactaaatgggaaggacatcggttggaatagttacagaaaggagctacaagatgacgagctgaagtctttgcaacgaggggcggagaccacttgggaccaaagcgaggacatggaatgggagagcgcagtggatgacatgaccaaaaagcaagtattcatttttgattctttggttaaaaagtgtctgtttgaagtgctcagcacaaagaacatagctcctagtgatgttacttggttcgtgcagcatgaatggggaaaggaccaaggctggcactgtcatgtgctgattggaggcaaggactttagtcaacctcaaggaaagtggtggagaaggcagctaaatgtgtactggagtagatggttggtgactgcctgtaatgttcaactaacaccagctgaaagaattaaactgagagaaatagcagaggacagtgaatgggtcactttgcttacctataagcataaacacaccaagaaggactataccaagtgtgttttttttggaaacatgattgcttattactttctaagcaaaaagaaaatatgtaccagtccaccaagggacggaggctattttcttagcagtgactctggctggaaaactaactttttgaaagagggcgagcgccatctagtgagcaaactgtatactgatgagatgaaaccagaaacggtcgagaccacagtgaccactgcgcaggaagctaagcgcggcagaattcaaactagaaaggaggtctcgattaaaaccacactcaaagagttggtgcataaaagagtaacctcaccagaagactggatgatgatgcagccagacagttacattgaaatgatggctcaaccaggtggagaaaacttgcttaaaaatacactagagatctgtacactgactctagcaagaaccaaaacagcctttgacttgattctagaaaaagctgaaaccagcaaactagccaacttttccatggctaacaccagaacctgtagaatctttgctgagcatggctggaactatattaaagtctgccatgccatctgttgtgtgctgaatagacaaggaggcaaaaggaacactgtgctctttcacggaccagccagcacaggcaaatctatcattgcacaagccatagcacaaggagttggtaatgttggttgttacaatgctgccaatgtgaactttccatttaatgactgtaccaacaaaaacttgatttgggtggaagaagctggtaactttggccagcaagtaaaccaattcaaagctatttgttctggccaaaccatacgcattgatcaaaaaggaaaaggcagcaaacagattgaaccaacaccagttatcatgaccaccaacgagaacattaccgtggtcagaataggctgtgaggaaaggccagaacacactcaaccaatcagagacagaatgctcaacattcacctgacacgtacactgcctggtgactttggtctggtggataagcacgaatggcctctgatctgtgcttggttggtgaagaatggttaccaatctaccatggcttgttactgtgctaaatggggcaaagttcctgattggtcagaggactgggcggagccgaagctagagactcctataaattcgctaggttcaatgcgctcaccatctctgactccgagaagtacgcctctcagccagaactacgctcttactccacttgcatcggaccttgcggacctagctctagagccttggagcacaccaaatactcctgttgcgggcactgcagcaagccagaacactggggaggctggtttcacagcctcccaaggtgctcaacggagcccaacctggtccgagatcgaggcggatctgagagcgtgcttcagccaggaacagctggagaaagacttcagcgattcactgaccttggactaa

SEQ ID NO: 32 - DNA, 2019 bp, H-1 parvovirus
atggctggaaacgcttactccgatgaggttttgggagtaaccaactggctgaaggacaaaagtagccaggaggtgttctcatttgtttttaaaaatgaaaacgtccaactaaatggaaaggacatcggttggaatagttacagaaaggagctacaagatgacgagctgaagtctctacaacgaggggcggagaccacttgggaccaaagcgaggacatggaatgggagagcgcagtggatgacatgaccaaaaagcaagtatttatttttgattctttggttaagaagtgtttgtttgaagtgctcagcacaaagaacatagctcctagtaatgttacttggttcgtgcagcatgaatggggaaaggaccaaggctggcactgtcatgtgctgattggaggcaaggactttagtcaacctcaaggaaaatggtggagaaggcagctaaatgtgtactggagtagatggttggtgactgcctgtaatgttcaactaacaccagctgaaagaattaaactgagagaaatagcagaggacagtgaatgggtcactttgcttacctataagcataagcacaccaagaaggactataccaagtgtgttctttttggaaacatgattgcttattactttttaagcaaaaagaaaatatgtaccagtccaccaagggacggaggctattttcttagcagtgactctggctggaaaactaactttttgaaagagggcgagcgccatctagtgagcaaactgtatactgatgagatgaaaccagaaacggtcgagaccacagtgaccactgcacaggaagctaagcgcggcagaattcaaactagaaaggaggtctcgattaaaaccacactcaaagagttggtacataaaagagtaacctcaccagaagactggatgatgatgcagccagacagttacattgaaatgatggctcaaccaggtggagaaaacttgcttaaaaatacactagagatctgtacactgactctagcaagaaccaaaacagcctttgacttgattctggaaaaagctgaaaccagcaaactagccaacttttccatggctagcaccagaacctgtagaatctttgctgagcatggctggaactatattaaagtctgccatgccatctgttgtgtgctgaatagacaaggaggcaaaaggaacactgtgctctttcacggaccagccagcacaggcaaatctattattgcacaagccatagcacaagcagttggtaatgttggttgttacaatgctgccaatgtgaactttccatttaatgactgtaccaacaaaaacttgatttgggtggaagaagctggtaactttggccagcaagtaaaccaattcaaagctatttgttctggccaaaccatacgcattgatcaaaaaggaaaaggcagcaaacagattgaaccaacaccagttattatgaccaccaacgagaacattaccgtggttagaataggctgtgaggaaagaccagaacacactcaaccaatcagagacagaatgctcaacattcacctgacacgtacactacctggtgactttggtttggtggataagcacgaatggcctctgatctgtgcttggttggtgaagaatggttaccaatctaccatggcttgttactgtgctaaatggggcaaagttcctgattggtcagaggactgggcggagccgaagctagacactcctataaattcgctaggttcaatgcgctcaccatctctgactccgagaagtacgcctctcagccaaaactacgctcttactccacttgcatcggaccttgcggacctagctctagagccttggagcacaccaaatactcctgttgcgggcactgcagcaagccaaaacactggggaggctggttccacagcctgccaaggtgctcaacggagcccaacctggtccgagatcgaggcggatttgagagcttgcttcagtcaagaacagttggagagcgacttcaacgaggagctgaccttggactaa

SEQ ID NO: 33 - DNA, 2019 bp, Rat minute virus isolate NTU1
atggctggaaacgcttactccgatgaagttttgggagcaaccaactggctaaaggacaaaagtagccaggaggtgttctcatttgtttttaaaaatgagaacgtccaactaaatgggaaggacatcggttggaatagttacagaaaggagctacaagatgacgagctgaagtctctacaacgaggggcggagaccacttgggaccaaagcgaggacatggaatgggagagcgcagtggatgacatgaccaaaaagcaagtattcatttttgattctttggttaagaagtgtttgtttgaagtgctcagcacaaagaacatagctcctagtgatgttacttggttcgtgcagcatgaatggggaaaggaccaaggctggcactgtcatgtgttgattggaggcaaggactttagtcaagctcaaggaaaatggtggagaaggcagctaaatgtgtactggagtagatggttggtgactgcctgtaatgttcaactaacaccagctgaaagaattaaactgagagaaatagcagaggacagtgaatgggtcactttgcttacctataagcataagcacaccaagaaggactataccaagtgtgttctttttggaaacatgattgcttattactttctaagcaaaaagaaaatatgtaccagtccaccaagggacggaggctattttcttagcagtgactctggctggaaaactaactttttgaaagagggcgagcgccatctagtgagcaaactgtatactgatgagatgaaaccagaaacggtcgagaccacagtgaccactgcacaggaagctaagcgcggcagaattcaaactagaaaggaggtctcgattaaaaccacactcaaagagttggtacataaaagagtaacctcaccagaagactggatgatgatgcagccagacagttatattgaaatgatggctcaaccaggtggagaaaacttgcttaaaaatacactagagatatgtacactgactctagcaagaaccaaaacagcctttgacttgattctggaaaaagctgaaaccagcaaactagccaacttttctatggctaacaccagaacctgtagaatctttgctgagcatggctggaactatattaaagtctgccatgccatctgttgtgtgctaaatagacaaggaggcaaaaggaacactgtgctctttcacggaccagccagcacaggcaaatctatcattgcacaagccatagcacaagcagttggtaatgttggttgttacaatgctgccaatgtgaactttccatttaatgactgtaccaacaaaaacttgatttgggtggaagaagctggtaactttggccagcaagtaaaccaattcaaagctatttgttctggccaaaccatacgcattgatcaaaaaggaaaaggcagcaaacagattgaaccaacaccagttatcatgaccaccaacgagaacattaccgtggtcagaataggctgtgaggaaagaccagaacacactcaaccaatcagagacagaatgctcaacattcacctgacacgtacactgcctggtgactttggtctggtggataagcacgaatggcctctgatctgtgcttggttggtgaagaatggttaccaatctacaatggcttgttactgtgctaaatggggcaaagttcctgattggtcagaagactgggcggagccgaagctagagactcctataaattcgctaggttcaatgcgctcaccatctctgactccgagaagtacgcctctcagccagaactacgctcttactccacttgcatcggaccttgcggacctagctctggagccttggagcacaccaaatactcctgttgcgggcactgcagcaagccagaacactggggaggctggtttcgcagcctgccaaggtgctcaacggagcccaacctggtccgagatagaagcagacttgagagcttgcttcagtcaagaacagttggagagcgacttcaacgaggaactgaccttggactaa

SEQ ID NO: 34 - DNA, 2019 bp, Parvovirus h-1
atggctggaaacgcttactccgatgaggttttgggagtaacaaactggctgaaggacaaaagtagccaggaggtgttctcatttgtttttaaaaatgaaaacgtccaactaaatggaaaggacatcggttggaatagttacagaaaggagctacaagatgacgagctgaagtctctacaacgaggggcggagaccacttgggaccaaagcgaggacatggaatgggagagcgcagtggatgacatgaccaaaaagcaagtatttatttttgattctttggttaagaagtgtttgtttgaagtgctcagcacaaagaacatagctcctagtaatgttacttggttcgtgcagcatgaatggggaaaggacccaggctggcactgtcatgtgctgattggaggcaaggactttagtcaacctcaaggaaaatggtggagaaggcagctaaatgtgtactggagtagatggttggtgactgcctgtaatgttcaactaacaccagctgaaagaattaaactgagagaaatagcagaggacagtgaatgggtcactttgcttacctataagcataagcacaccaagaaggactataccaagtgtgttctttttggaaacatgattgcttattactttttaagcaaaaagaaaatatgtaccagtccaccaagggacggaggctattttcttagcagtgactctggctggaaaactaactttttgaaagagggcgagcgccatctagtgagcaaactgtatactgatgagatgaaaccagaaacggtcgagaccacagtgaccactgcacaggaagctaagcgcggcagaattcaaactagagaggaggtctcgattaaaaccacactcaaagagttggtacataaaagagtaacctcaccagaagactggatgatgatgcagccagacagttacattgaaatgatggctcaaccaggtggagaaaacttgcttaaaaatacactagagatctgtacactgactctagcaagaaccaaaacagcctttgacttgattctggaaaaagctgaaaccagcaaactagccaacttttccatggctagcaccagaacctgtagaatctttgctgagcatggctggaactatattaaagtctgccatgccatctgttgtgtgctgaatagacaaggaggcaaaaggaacactgtgctctttcacggaccagccagcacaggcaaatctattattgcacaagccatagcacaagcagttggtaatgttggttgttacaatgctgccaatgtgaactttccatttaatgactgtaccaacaaaaacttgatttgggtggaagaagctggtaactttggccagcaagtaaaccaattcaaagctatttgttctggccaaaccatacgcattgatcaaaaaggaaaaggcagcaaacagattgaaccaacaccagttattatgaccaccaacgagaacattaccgtggttagaataggctgtgaggaaagaccagaacacactcaaccaatcagagacagaatgctcaacattcacctgacacgtacactacctggtgactttggtttggtggataagcacgaatggcctctgatctgtgcttggttggtgaagaatggttaccaatctaccatggcttgttactgtgctaaatggggcaaagttcctgattggtcagaggactgggcggagccgaagctagacactcctataaattcgctaggttcaatgcgctcaccatctctgactccgagaagtacgcctctcagccaaaactacgctcttactccacttgcatcggaccttgcggacctagctctagagccttggagcacaccaaatactcctgttgcgggcactgcagcaagccaaaacactggggaggctggttccacagcctgccaaggtgctcaacggagcccaacctggtccgagatcgaggcggatttgagagcttgcttcagtcaagaacagttggagagcgacttcaacgaggagctgaccttggactaa

SEQ ID NO: 35 - DNA, 1997 bp, Rat minute virus isolate NTU2
atgaggttttgggagcaaccaactggctaaaggacaaaagtagccaggaggtattctcatttgtttttaaaaatgagaacgtccaactaaatgggaaggacatcggttggaatagttacagaaaggagctacaagatgacgagctgaagtctctacaacgaggggcggagaccacttgggaccaaagcgaggacatggaatgggagagcgcagtggatgacatgaccaaaaagcaagtattcatttttgattctttggttaagaagtgtctgtttgaagtgctcagcacaaagaacatagctcctagtgatgttacttggttcgtgcagcatgaatggggaaaggaccaaggctggcactgtcatgtgctgattggaggcaaggactttagtcaagctcaaggaaaatggtggagaaggcagctaaatgtgtactggagtagatggttggtgactgcctgtaatgttcaactaacaccagctgaaagaattaaactaagagaaatagcagaggacagtgaatgggtcactttgcttacctataagcataagcacaccaagaaggactataccaagtgtgttctttttggaaacatgattgcttattactttctaagcaaaaagaaaatatgtaccagtccaccaagggacggaggctattttcttagcagtgactctggctggaaaactaactttttgaaagagggcgagcgccatctagtgagcaaactgtatactgatgagatgaaaccagaaacggtcgagaccacagtgaccactgcacaggaagctaagcgcggcagaattcaaactagaaaggaggtctcgattaaaaccacactcaaagagttggtacataaaagagtaacctcaccagaagactggatgatgatgcagccagacagttatattgaaatgatggctcaaccaggtggagaaaacttgcttaaaaatacactagagatatgtacactgactctagcaagaaccaaaacagcctttgacttgattctggaaaaagctgaaaccagcaaactagccaacttttctatggctagcaccagaacctgtagaatctttgctgagcatggctggaactatattaaagtctgccatgccatctgttgtgtgctaaatagacaaggaggcaaaaggaacactgtgctctttcacggaccagccagcacaggcaaatctatcattgcacaagccatagcacaagcagttggtaatgttggttgttacaatgctgccaatgtgaactttccatttaatgactgtaccaacaaaaacttgatttgggtggaagaagctggtaactttggccagcaagtaaaccaattcaaagctatttgttctggccaaaccatacgcattgatcaaaaaggaaaaggcagcaaacagattgaaccaacaccagttatcatgaccaccaacgagaacattaccgtggtcagaataggctgtgaggaaagaccagaacacactcaaccaatcagagacagaatgctcaacattcacctgacacgtacactgcctggtgactttggtctggtggataagcacgaatggcctctgatctgtgcttggttggtgaagaatggttaccaatctaccatggcttgttactgtgctaaatggggcaaagttcctgattggtcagaagactgggcggagccgaagctagagactcctataaattcgctaggttcaatgcgctcaccatctctgactccgagaagtacgcctctcagccagaactacgctcttactccacttgtatcggaccttgcggacctagctctggagccttggagcacaccaaatactcctgttgcgggcactgcagcaagccagaacactggggaggctggtttcgcagcctgtcaaggtgctcaacggagcccaacctggtccgagatagaagcagacttgagagcttgcttcagtcaagaacagttggagagcgacttcaacgaggagctgaccttggactaa

SEQ ID NO: 36 - DNA, 2019 bp, Rat minute virus 2a
atggctggaaacgcttactccgatgaggttttgggagcaaccaactggctaaaggacaaaagtagccaggaggtgttctcatttgtttttaaaaatgagaacgtccaactaaatgggaaggacatcggttggaatagttacagaaaggagctacaagatgacgagctgaagtctctacaacgaggggcggagaccacttgggaccaaagcgaggacatggaatgggagagcgcagtggatgacatgaccaaaaagcaagtattcatttttgattctttggttaagaagtgtctgtttgaagtgctcagcacaaagaacatagctcctagtgatgttacttggttcgtgcagcatgaatggggaaaggaccaaggctggcactgtcatgtgctgattggaggcaaggactttagtcaagctcaaggaaaatggtggagaaggcagctaaatgtgtactggagtagatggttggtgactgcctgtaatgttcaactaacaccagctgaaagaattaaactgagagaaatagcagaggacagtgaatgggtcactttgcttacctataagcataagcacaccaagaaggactataccaagtgtgttctttttggaaacatgattgcttattactttctaagcaaaaagaaaatatgtaccagtccaccaagggacggaggctattttcttagcagtgactctggctggaaaactaacttcttgaaagagggcgagcgccatctagtgagcaaactgtatactgatgagatgaaaccagaaacggtcgagaccacagtgaccactgcgcaggaagctaagcgcggcagaattcaaactagaaaggaggtctcgattaaaaccacactcaaagagttggtgcataaaagagtaacctcaccagaagactggatgatgatgcagccagacagttacattgaaatgatggctcaaccaggtggagaaaacttgcttaaaaatacactagagatatgtacactgactctagcaagaaccaaaacagcctttgacttgattctggaaaaagctgaaaccagcaaactagccaacttttccatggctagcaccagaacctgtagaatctttgttgagcatggctggaactatattaaagtctgccatgccatctgttgtgtactaaatagacaaggaggcaaaaggaacactgtgctctttcacggaccagccagcacaggcaaatctatcattgcacaagccatagcacaagcagttggtaatgttggttgttacaatgctgccaatgtgaactttccatttaatgactgtaccaacaaaaacttgatttgggtggaagaagctggtaactttggccagcaagtaaaccaattcaaagctatttgttctggccaaaccatacgcattgatcaaaaaggaaaaggcagcaaacagattgaaccaacaccagttatcatgaccaccaacgaaaacattaccgtggtcagaataggctgtgaggaaagaccagaacacactcaaccaatcagagacagaatgctcaacattcacctgacacgtacactgcctggtgactttggtctggtggataagcacgaatggcctctgatctgtgcttggttggtgaagaatggttaccaatctacaatggcttgttactgtgctaaatggggcaaagttcctgattggtcagaagactgggcggagccgaagctagagactcctataaattcgctaggttcaatgcgctcaccatctctgactccgagaagtacgcctctcagccagaactacgctcttactccacttgcatcggaccttgcggacctagctctggagccttggagcacaccaaatactcctgttgcgggcactgtagcaagccagaacactggggaggctggtttcgcagcctgccaaggtgctcaacggagcccaacctggtccgagatagaagcagacttgagagcttgcttcagtcaagaacagttggagagcgacttcaacgaggaactgaccttggactaa

SEQ ID NO: 37 - DNA, 192 bp, Artificial
  consensus sequence
ctarrrargargtytcdattaaaacyacactyaaagarytrgtrcataaragagtaacctcaccagargactggatgatgatgcagccagacagttayattgaaatgatggctcarccaggkggagaaaacytrctdaaraatacrctagaratytgtacrctractctagchagaacmaaaacagcmtttg